European Patent Application EP 4 163 368 A1, published April 12, 2023. Title: Ketoreductase Mutant and Applications thereof. Applicant: ASYMCHEM LIFE SCIENCE(TIANJIN)CO.,LTD. The sequence listing filed with the application follows.

SEQUENCE LISTING (1 sequence)

SEQ ID NO: 1 - protein, 253 aa, Acetobacter pasteurianus
MARVAGKVAIVSGAANGIGKATAQLLAKEGAKVVIGDLKEEDGQKAVAEIKAAGGEAAFVKLNVTDEAAWKAAIGQTLKLYGRLDIAVNNAGITYSGSVESTSLEDWRRVQSINLDGVFLGTQVAIEAMKKSGGGSIVNLSSIEGLIGDPMLAAYNASKGGVRLFTKSAALHCAKSGYKIRVNSVHPGYIWTPMVAGLTKEDAAARQKLVDLHPIGHLGEPNDIAYGILYLASDESKFVTGSELVIDGGYTAQ